European Patent Application EP 4 342 478 A1, published March 27, 2024. Title: Prophylaxis and/or treatment agent for pressure ulcer. Applicant: Cysay Inc. Tokyo Medical University. The sequence listing filed with the application follows.

SEQUENCE LISTING (19 sequences)

SEQ ID NO: 1 - DNA, 1978 bp, Artificial Sequence
  DNA fragment for gene transduction
  misc_feature (1)..(1978): SYN122-1-7
  misc_feature (1)..(1978): SYN4122-1-7
agctgacgtggaagatgagcgtgcgggactgcgcttggctgcgcaggagcccaggggttggctgtgttccggccgcagagcaccgtctgcgtgaggagatcctggccaagttcctgcactggctgatgagtgtgtacgtcgtcgagctgctcaggtctttcttttatgtcacggagaccacgtttcaaaagaacaggctctttttctaccggaagagtgtctggagcaagttgcaaagcattggaatcagacagcacttgaagagggtgcagctgcgggagctgtcggaagcagaggtcaggcagcatcgggaagccaggcccgccctgctgacgtccagactccgcttcatccccaagcctgacgggctgcggccgattgtgaacatggactacgtcgtgggagccagaacgttccgcagagaaaagagggccgagcgtctcacctcgagggtgaaggcactgttcagcgtgctcaactacgagcgggcgcggcgccccggcctcctgggcgcctctgtgctgggcctggacgatatccacagggcctggcgcaccttcgtgctgcgtgtgcgggcccaggacccgccgcctgagctgtactttgtcaaggtggatgtgacgggcgcgtacgacaccatcccccaggacaggctcacggaggtcatcgccagcatcatcaaaccccagaacacgtactgcgtgcgtcggtatgccgtggtccagaaggccgcccatgggcacgtccgcaaggccttcaagagccacgtctctaccttgacagacctccagccgtacatgcgacagttcgtggctcacctgcaggagaccagcccgctgagggatgccgtcgtcatcgagcagagctcctccctgaatgaggccagcagtggcctcttcgacgtcttcctacgcttcatgtgccaccacgccgtgcgcatcaggggcaagtcctacgtccagtgccaggggatcccgcagggctccatcctctccacgctgctctgcagcctgtgctacggcgacatggagaacaagctgtttgcggggattcggcgggacgggctgctcctgcgtttggtggatgatttcttgttggtgacacctcacctcacccacgcgaaaaccttcctcaggaccctggtccgaggtgtccctgagtatggctgcgtggtgaacttgcggaagacagtggtgaacttccctgtagaagacgaggccctgggtggcacggcttttgttcagatgccggcccacggcctattcccctggtgcggcctgctgctggatacccggaccctggaggtgcagagcgactactccagctatgcccggacctccatcagagccagtctcaccttcaaccgcggcttcaaggctgggaggaacatgcgtcgcaaactctttggggtcttgcggctgaagtgtcacagcctgtttctggatttgcaggtgaacagcctccagacggtgtgcaccaacatctacaagatcctcctgctgcaggcgtacaggtttcacgcatgtgtgctgcagctcccatttcatcagcaagtttggaagaaccccacatttttcctgcgcgtcatctctgacacggcctccctctgctactccatcctgaaagccaagaacgcagggatgtcgctgggggccaagggcgccgccggccctctgccctccgaggccgtgcagtggctgtgccaccaagcattcctgctcaagctgactcgacaccgtgtcacctacgtgccactcctggggtcactcaggacagcccagacgcagctgagtcggaagctcccggggacgacgctgactgccctggaggccgcagccaacccggcactgccctcagacttcaagaccatcctggactgaggatccaattctaccgggtaggggaggcgcttttcccaaggcagtctggagcatgcgctttagcagccccgctgggcacttggcgctacacaagtggc

SEQ ID NO: 2 - DNA, 2556 bp, Artificial Sequence
  DNA fragment for gene transduction
  misc_feature (1)..(2556): SYN4122-2-2
ccatccacgctgttttgacctccatagaagacaccgactctactagaggatctatttccggtgaattcgccacccatcgaacaacgagaatcaagatcactgagctaaatccccacctgatgtgtgtgctttgtggagggtacttcattgatgccacaaccataatagaatgtctacattccttctgtaaaacgtgtattgttcgttacctggagaccagcaagtattgtcctatttgtgatgtccaagttcacaagaccagaccactactgaatataaggtcagataaaactctccaagatattgtatacaaattagttccagggcttttcaaaaatgaaatgaagagaagaagggatttttatgcagctcatccttctgctgatgctgccaatggctctaatgaagatagaggagaggttgcagatgaagataagagaattataactgatgatgagataataagcttatccattgaattctttgaccagaacagattggatcggaaagtaaacaaagacaaagagaaatctaaggaggaggtgaatgataaaagatacttacgatgcccagcagcaatgactgtgatgcacttaagaaagtttctcagaagtaaaatggacatacctaatactttccagattgatgtcatgtatgaggaggaacctttaaaggattattatacactaatggatattgcctacatttatacctggagaaggaatggtccacttccattgaaatacagagttcgacctacttgtaaaagaatgaagatcagtcaccagagagatggactgacaaatgctggagaactggaaagtgactctgggagtgacaaggccaacagcccagcaggaggtattccctccacctcttcttgtttgcctagccccagtactccagtgcagtctcctcatccacagtttcctcacatttccagtactatgaatggaaccagcaacagccccagcggtaaccaccaatcttcttttgccaatagacctcgaaaatcatcagtaaatgggtcatcagcaacttcttctggtggatctgaaggtaggggaagtttgcttacttgcggtgacgtcgaagagaatccaggaccagatggccgcaacatgccgcgcgctccccgctgccgagccgtgcgctccctgctgcgcagccactaccgcgaggtgctgccgctggccacgttcgtgcggcgcctggggccccagggctggcggctggtgcagcgcggggacccggcggctttccgcgcgctggtggcccagtgcctggtgtgcgtgccctgggacgcacggccgccccccgccgccccctccttccgccaggtgtcctgcctgaaggagctggtggcccgagtgctgcagaggctgtgcgagcgcggcgcgaagaacgtgctggccttcggcttcgcgctgctggacggggcccgcgggggcccccccgaggccttcaccaccagcgtgcgcagctacctgcccaacacggtgaccgacgcactgcgggggagcggggcgtgggggctgctgctgcgccgcgtgggcgacgacgtgctggttcacctgctggcacgctgcgcgctctttgtgctggtggctcccagctgcgcctaccaggtgtgcgggccgccgctgtaccagctcggcgctgccactcaggcccggcccccgccacacgctagtggaccccgaaggcgtctgggatgcgaacgggcctggaaccatagcgtcagggaggccggggtccccctgggcctgccagccccgggtgcgaggaggcgcgggggcagtgccagccgaagtctgccgttgcccaagaggcccaggcgtggcgctgcccctgagccggagcggacgcccgttgggcaggggtcctgggcccacccgggcaggacgcgtggaccgagtgaccgtggtttctgtgtggtgtcacctgccagacccgccgaagaagccacctctttggagggtgcgctctctggcacgcgccactcccacccatccgtgggccgccagcaccacgcgggccccccatccacatcgcggccaccacgtccctgggacacgccttgtcccccggtgtacgccgagaccaagcacttcctctactcctcaggcgacaaggagcagctgcggccctccttcctactcagctctctgaggcccagcctgactggcgctcggaggctcgtggagaccatctttctgggttccaggccctggatgccagggactccccgcaggttgccccgcctgccccagcgctactggcaaatgcggcccctgtttctggagctgcttgggaaccacgcgcagtgcccctacggggtgctcctcaagacgcactgcccgctgcgagctgcggtcaccccagcagccggtgtctgtgcccgggagaagccccagggctctgtggcggcccccgaggaggaggacacagacccccgtcgcctggtgcagctgctccgccagcacagcagcccctggcaggtgtacggcttcgtgcgggcctgcctgcgccggctggtgcccccaggcctctggg

SEQ ID NO: 3 - DNA, 2983 bp, Artificial Sequence
  DNA fragment for gene transduction
  misc_feature (1)..(2983): SYN4122-3-3
ccacgctgttttgacctccatagaagacaccgactctactagaggatctatttccggtgaattcgccacccatcgaacaacgagaatcaagatcactgagctaaatccccacctgatgtgtgtgctttgtggagggtacttcattgatgccacaaccataatagaatgtctacattccttctgtaaaacgtgtattgttcgttacctggagaccagcaagtattgtcctatttgtgatgtccaagttcacaagaccagaccactactgaatataaggtcagataaaactctccaagatattgtatacaaattagttccagggcttttcaaaaatgaaatgaagagaagaagggatttttatgcagctcatccttctgctgatgctgccaatggctctaatgaagatagaggagaggttgcagatgaagataagagaattataactgatgatgagataataagcttatccattgaattctttgaccagaacagattggatcggaaagtaaacaaagacaaagagaaatctaaggaggaggtgaatgataaaagatacttacgatgcccagcagcaatgactgtgatgcacttaagaaagtttctcagaagtaaaatggacatacctaatactttccagattgatgtcatgtatgaggaggaacctttaaaggattattatacactaatggatattgcctacatttatacctggagaaggaatggtccacttccattgaaatacagagttcgacctacttgtaaaagaatgaagatcagtcaccagagagatggactgacaaatgctggagaactggaaagtgactctgggagtgacaaggccaacagcccagcaggaggtattccctccacctcttcttgtttgcctagccccagtactccagtgcagtctcctcatccacagtttcctcacatttccagtactatgaatggaaccagcaacagccccagcggtaaccaccaatcttcttttgccaatagacctcgaaaatcatcagtaaatgggtcatcagcaacttcttctggtggatctgaaggcagaggctctctgctgacatgtggggatgtggaggaaaatcctggccctacgcgtcaccaaaagagaactgcaatgtttcaggacccacaggagcgacccagaaagttaccacagttatgcacagagctgcaaacaactatacatgatataatattagaatgtgtgtactgcaagcaacagttactgcgacgtgaggtatatgactttgcttttcgggatttatgcatagtatatagagatgggaatccatatgctgtatgtgataaatgtttaaagttttattctaaaattagtgagtatagacattattgttatagtttgtatggaacaacattagaacagcaatacaacaaaccgttgtgtgatttgttaattaggtgtattaactgtcaaaagccactgtgtcctgaagaaaagcaaagacatctggacaaaaagcaaagattccataatataaggggtcggtggaccggtcgatgtatgtcttgttgcagatcatcaagaacacgtagagaaacccagctgggatctgaaggtaggggaagtttgcttacttgcggtgacgtcgaagagaatccaggaccagatggccgcaacatgccgcgcgctccccgctgccgagccgtgcgctccctgctgcgcagccactaccgcgaggtgctgccgctggccacgttcgtgcggcgcctggggccccagggctggcggctggtgcagcgcggggacccggcggctttccgcgcgctggtggcccagtgcctggtgtgcgtgccctgggacgcacggccgccccccgccgccccctccttccgccaggtgtcctgcctgaaggagctggtggcccgagtgctgcagaggctgtgcgagcgcggcgcgaagaacgtgctggccttcggcttcgcgctgctggacggggcccgcgggggcccccccgaggccttcaccaccagcgtgcgcagctacctgcccaacacggtgaccgacgcactgcgggggagcggggcgtgggggctgctgctgcgccgcgtgggcgacgacgtgctggttcacctgctggcacgctgcgcgctctttgtgctggtggctcccagctgcgcctaccaggtgtgcgggccgccgctgtaccagctcggcgctgccactcaggcccggcccccgccacacgctagtggaccccgaaggcgtctgggatgcgaacgggcctggaaccatagcgtcagggaggccggggtccccctgggcctgccagccccgggtgcgaggaggcgcgggggcagtgccagccgaagtctgccgttgcccaagaggcccaggcgtggcgctgcccctgagccggagcggacgcccgttgggcaggggtcctgggcccacccgggcaggacgcgtggaccgagtgaccgtggtttctgtgtggtgtcacctgccagacccgccgaagaagccacctctttggagggtgcgctctctggcacgcgccactcccacccatccgtgggccgccagcaccacgcgggccccccatccacatcgcggccaccacgtccctgggacacgccttgtcccccggtgtacgccgagaccaagcacttcctctactcctcaggcgacaaggagcagctgcggccctccttcctactcagctctctgaggcccagcctgactggcgctcggaggctcgtggagaccatctttctgggttccaggccctggatgccagggactccccgcaggttgccccgcctgccccagcgctactggcaaatgcggcccctgtttctggagctgcttgggaaccacgcgcagtgcccctacggggtgctcctcaagacgcactgcccgctgcgagctgcggtcaccccagcagccggtgtctgtgcccgggagaagccccagggctctgtggcggcccccgaggaggaggacaca

SEQ ID NO: 4 - DNA, 2223 bp, Artificial Sequence
  DNA fragment for gene transduction
  misc_feature (1)..(2223): SYN4122-4-4
acgctgttttgacctccatagaagacaccgactctactagaggatctatttccggtgaattcgccacccaccaaaagagaactgcaatgtttcaggacccacaggagcgacccagaaagttaccacagttatgcacagagctgcaaacaactatacatgatataatattagaatgtgtgtactgcaagcaacagttactgcgacgtgaggtatatgactttgcttttcgggatttatgcatagtatatagagatgggaatccatatgctgtatgtgataaatgtttaaagttttattctaaaattagtgagtatagacattattgttatagtttgtatggaacaacattagaacagcaatacaacaaaccgttgtgtgatttgttaattaggtgtattaactgtcaaaagccactgtgtcctgaagaaaagcaaagacatctggacaaaaagcaaagattccataatataaggggtcggtggaccggtcgatgtatgtcttgttgcagatcatcaagaacacgtagagaaacccagctgggatctgaaggcagaggctctctgctgacatgtggggatgtggaggaaaatcctggccctacgcgtcatggagatacacctacattgcatgaatatatgttagatttgcaaccagagacaactgatctctactgttatgagcaattaaatgacagctcagaggaggaggatgaaatagatggtccagctggacaagcagaaccggacagagcccattacaatattgtaaccttttgttgcaagtgtgactctacgcttcggttgtgcgtacaaagcacacacgtagacattcgtactttggaagacctgttaatgggcacactaggaattgtgtgccccatctgttctcagaaaccaggatctgaaggtaggggaagtttgcttacttgcggtgacgtcgaagagaatccaggaccagatggccgcaacatgccgcgcgctccccgctgccgagccgtgcgctccctgctgcgcagccactaccgcgaggtgctgccgctggccacgttcgtgcggcgcctggggccccagggctggcggctggtgcagcgcggggacccggcggctttccgcgcgctggtggcccagtgcctggtgtgcgtgccctgggacgcacggccgccccccgccgccccctccttccgccaggtgtcctgcctgaaggagctggtggcccgagtgctgcagaggctgtgcgagcgcggcgcgaagaacgtgctggccttcggcttcgcgctgctggacggggcccgcgggggcccccccgaggccttcaccaccagcgtgcgcagctacctgcccaacacggtgaccgacgcactgcgggggagcggggcgtgggggctgctgctgcgccgcgtgggcgacgacgtgctggttcacctgctggcacgctgcgcgctctttgtgctggtggctcccagctgcgcctaccaggtgtgcgggccgccgctgtaccagctcggcgctgccactcaggcccggcccccgccacacgctagtggaccccgaaggcgtctgggatgcgaacgggcctggaaccatagcgtcagggaggccggggtccccctgggcctgccagccccgggtgcgaggaggcgcgggggcagtgccagccgaagtctgccgttgcccaagaggcccaggcgtggcgctgcccctgagccggagcggacgcccgttgggcaggggtcctgggcccacccgggcaggacgcgtggaccgagtgaccgtggtttctgtgtggtgtcacctgccagacccgccgaagaagccacctctttggagggtgcgctctctggcacgcgccactcccacccatccgtgggccgccagcaccacgcgggccccccatccacatcgcggccaccacgtccctgggacacgccttgtcccccggtgtacgccgagaccaagcacttcctctactcctcaggcgacaaggagcagctgcggccctccttcctactcagctctctgaggcccagcctgactggcgctcggaggctcgtggagaccatctttctgggttccaggccctggatgccagggactccccgcaggttgccccgcctgccccagcgctactggcaaatgcggcccctgtttctggagctgcttgggaaccacgcgcagtgcccctacggggtgctcctcaagacgcactgcccgctgcgagctgcgg

SEQ ID NO: 5 - DNA, 3399 bp, Homo sapiens
  misc_feature: hTERT
  gene (1)..(3399): hTERT
atgccgcgcgctccccgctgccgagccgtgcgctccctgctgcgcagccactaccgcgaggtgctgccgctggccacgttcgtgcggcgcctggggccccagggctggcggctggtgcagcgcggggacccggcggctttccgcgcgctggtggcccagtgcctggtgtgcgtgccctgggacgcacggccgccccccgccgccccctccttccgccaggtgtcctgcctgaaggagctggtggcccgagtgctgcagaggctgtgcgagcgcggcgcgaagaacgtgctggccttcggcttcgcgctgctggacggggcccgcgggggcccccccgaggccttcaccaccagcgtgcgcagctacctgcccaacacggtgaccgacgcactgcgggggagcggggcgtgggggctgctgctgcgccgcgtgggcgacgacgtgctggttcacctgctggcacgctgcgcgctctttgtgctggtggctcccagctgcgcctaccaggtgtgcgggccgccgctgtaccagctcggcgctgccactcaggcccggcccccgccacacgctagtggaccccgaaggcgtctgggatgcgaacgggcctggaaccatagcgtcagggaggccggggtccccctgggcctgccagccccgggtgcgaggaggcgcgggggcagtgccagccgaagtctgccgttgcccaagaggcccaggcgtggcgctgcccctgagccggagcggacgcccgttgggcaggggtcctgggcccacccgggcaggacgcgtggaccgagtgaccgtggtttctgtgtggtgtcacctgccagacccgccgaagaagccacctctttggagggtgcgctctctggcacgcgccactcccacccatccgtgggccgccagcaccacgcgggccccccatccacatcgcggccaccacgtccctgggacacgccttgtcccccggtgtacgccgagaccaagcacttcctctactcctcaggcgacaaggagcagctgcggccctccttcctactcagctctctgaggcccagcctgactggcgctcggaggctcgtggagaccatctttctgggttccaggccctggatgccagggactccccgcaggttgccccgcctgccccagcgctactggcaaatgcggcccctgtttctggagctgcttgggaaccacgcgcagtgcccctacggggtgctcctcaagacgcactgcccgctgcgagctgcggtcaccccagcagccggtgtctgtgcccgggagaagccccagggctctgtggcggcccccgaggaggaggacacagacccccgtcgcctggtgcagctgctccgccagcacagcagcccctggcaggtgtacggcttcgtgcgggcctgcctgcgccggctggtgcccccaggcctctggggctccaggcacaacgaacgccgcttcctcaggaacaccaagaagttcatctccctggggaagcatgccaagctctcgctgcaggagctgacgtggaagatgagcgtgcgggactgcgcttggctgcgcaggagcccaggggttggctgtgttccggccgcagagcaccgtctgcgtgaggagatcctggccaagttcctgcactggctgatgagtgtgtacgtcgtcgagctgctcaggtctttcttttatgtcacggagaccacgtttcaaaagaacaggctctttttctaccggaagagtgtctggagcaagttgcaaagcattggaatcagacagcacttgaagagggtgcagctgcgggagctgtcggaagcagaggtcaggcagcatcgggaagccaggcccgccctgctgacgtccagactccgcttcatccccaagcctgacgggctgcggccgattgtgaacatggactacgtcgtgggagccagaacgttccgcagagaaaagagggccgagcgtctcacctcgagggtgaaggcactgttcagcgtgctcaactacgagcgggcgcggcgccccggcctcctgggcgcctctgtgctgggcctggacgatatccacagggcctggcgcaccttcgtgctgcgtgtgcgggcccaggacccgccgcctgagctgtactttgtcaaggtggatgtgacgggcgcgtacgacaccatcccccaggacaggctcacggaggtcatcgccagcatcatcaaaccccagaacacgtactgcgtgcgtcggtatgccgtggtccagaaggccgcccatgggcacgtccgcaaggccttcaagagccacgtctctaccttgacagacctccagccgtacatgcgacagttcgtggctcacctgcaggagaccagcccgctgagggatgccgtcgtcatcgagcagagctcctccctgaatgaggccagcagtggcctcttcgacgtcttcctacgcttcatgtgccaccacgccgtgcgcatcaggggcaagtcctacgtccagtgccaggggatcccgcagggctccatcctctccacgctgctctgcagcctgtgctacggcgacatggagaacaagctgtttgcggggattcggcgggacgggctgctcctgcgtttggtggatgatttcttgttggtgacacctcacctcacccacgcgaaaaccttcctcaggaccctggtccgaggtgtccctgagtatggctgcgtggtgaacttgcggaagacagtggtgaacttccctgtagaagacgaggccctgggtggcacggcttttgttcagatgccggcccacggcctattcccctggtgcggcctgctgctggatacccggaccctggaggtgcagagcgactactccagctatgcccggacctccatcagagccagtctcaccttcaaccgcggcttcaaggctgggaggaacatgcgtcgcaaactctttggggtcttgcggctgaagtgtcacagcctgtttctggatttgcaggtgaacagcctccagacggtgtgcaccaacatctacaagatcctcctgctgcaggcgtacaggtttcacgcatgtgtgctgcagctcccatttcatcagcaagtttggaagaaccccacatttttcctgcgcgtcatctctgacacggcctccctctgctactccatcctgaaagccaagaacgcagggatgtcgctgggggccaagggcgccgccggccctctgccctccgaggccgtgcagtggctgtgccaccaagcattcctgctcaagctgactcgacaccgtgtcacctacgtgccactcctggggtcactcaggacagcccagacgcagctgagtcggaagctcccggggacgacgctgactgccctggaggccgcagccaacccggcactgccctcagacttcaagaccatcctggactga

SEQ ID NO: 6 - DNA, 477 bp, Human papillomavirus type 16
  gene (1)..(477): HPV16 E6
atgcaccaaaagagaactgcaatgtttcaggacccacaggagcgacccagaaagttaccacagttatgcacagagctgcaaacaactatacatgatataatattagaatgtgtgtactgcaagcaacagttactgcgacgtgaggtatatgactttgcttttcgggatttatgcatagtatatagagatgggaatccatatgctgtatgtgataaatgtttaaagttttattctaaaattagtgagtatagacattattgttatagtttgtatggaacaacattagaacagcaatacaacaaaccgttgtgtgatttgttaattaggtgtattaactgtcaaaagccactgtgtcctgaagaaaagcaaagacatctggacaaaaagcaaagattccataatataaggggtcggtggaccggtcgatgtatgtcttgttgcagatcatcaagaacacgtagagaaacccagctgtaa

SEQ ID NO: 7 - DNA, 297 bp, Human papillomavirus type 16
  gene (1)..(297): HPV 16 E7
atgcatggagatacacctacattgcatgaatatatgttagatttgcaaccagagacaactgatctctactgttatgagcaattaaatgacagctcagaggaggaggatgaaatagatggtccagctggacaagcagaaccggacagagcccattacaatattgtaaccttttgttgcaagtgtgactctacgcttcggttgtgcgtacaaagcacacacgtagacattcgtactttggaagacctgttaatgggcacactaggaattgtgtgccccatctgttctcagaaaccataa

SEQ ID NO: 8 - DNA, 3396 bp, swine
  gene (1)..(3396): pigTERT
atgccgcgcgcgccccggtgccgggccgtgcgctccctgctccgggaccgctacaggcaggtgctgccgctggccaccttcgtgcggcgcctgggccctgagggccggcggcttgttcggcgcggggacccggcggcctaccgcgcgctggtggcgcagtgcctggtgtgcgtgccctgggacgcgcagccgcctcctgcctccccgtccttccgccaggtgtcctgcctgaaggagctggtggccagggtcgtgcagaggctctgcgagcgcggcgcgaggaacgtgctggcctttggcttcgcgctgctggacggggctcgcggcgggccgcccgtggccttcacgaccagcgtgcgcagctacctgcccaacaccgtgaccgacacactgcgcgggagcggcgcgtgggggctgctgctgcgccgcgtgggcgacgacgtgctcacccacctgttggcgcgctgcgcgctgtacctgctggtgcccccgagttgcgcctaccaggtgtgcgggccgccactctatgacctctacaccgcagcggaggctcggcccatgcgacacaagggccagaccccgactggcctcggactcacgcgccccgtttgcaatggggaagccgggcgaccccaggagcagagggcgcaaggtgtgaggcgacgtcggggcagagcggggggacatccacttccagccaagaggcccaggcacgtcccggagcctgaacagggtcccgaagggcaggcgtcccgggcccaccagggcagggcgcctgggccgagcgacagcgacccccccgtgatgacacctaccagagccgctgcgaaagccaagtctcgggagggtgaggcgcccggaacccggcacctttcccctcaagcaggcggtgcgcggggtacctgccccccatcctggtggcagccacacctccagggcaagcccagtcctcatgtgtgcgctgccgagaccaagcgcttcctctactgctcggggagcaaggaagggctgcgccgctcgttcctgctctgctccctgccgcccagcctggcgggggccgggaggctcgtggaggtcatctttctggcctcaaagcccgggcagccaggggcgcgccgcgtgcccgcacgctactggcggatgaggcccctgttccgggagctgcttaagaaccacgcgcggtgcccctacaaggcgcttctcagggcgcactgcccgttgcgggctgcggcgaccctctcggggtccggcggtcaggtgtgcgaccacaaagtgggccccctcgctccagagcggctggcagcggccgccgagggggactcggcctcgaggcgcctagtccagctgctccgccagcacagcagcccctggcaggtgtaccgcctcctgcgggcctgtcttcaccggctggtgcccccgggcctctggggctccccgcacaacaagcggcgctttctgaagaatgtgaagaagctcgtctccctggggaagcacgccaggctctcgctgcaggagctgatgtggaagatgaaagtgcaagactgcatctggctgcgccggagcccggacgctcgccatgtccaggccgccgagcaccgtctgagagaggccattctggccaagttcctgcgctggttgatgggcacgtacgtggtcgagctgctcaggtcgtttttttatgtcacggagaccacgtttcagaagaaccggctcttcttcttccggaagcgcatctggagccggctgcagagcgcaggcatcaggcaacacttagatcgtgtgcggcttcgagaactgtcggaagcagagatcaggcgacgccgggaggccaggcccgctgtactgacctccaagctccgcttcgtccccaaacccgacgggctgcggcccatcgtgaacatggcgaacgtcgtgcgagccaggacaggccccggagacaagaaggtccggcgtctcacggggcaggtcaagacgctgtttgctgtgctgaactacgagcgggcgcggcgcccgcgcctcctgggggcctccgtgctgggcgtgggtgacatccacagggcgtggcgggcctttgtgctgcccctgcgggcccaggacccggcccccccgctgtactttgtcaaggtggacgtgacgggggcctacgacgccctccctcaggacaggcttgctgaggtggtcgccaacgtgatccggccctacgagagcacgtactgcgtgcgccagtgcgccgtgctccggaggaccgcccgcgggcacgtgcgcaagtccttccaaacccacgtgtccaccttcgcagacctccagccttacatgagacagtttgtggcacacctgcaggcaaccggcccgctgagggacgccgtggtcatcgagcagagctgctctctgaacgaggccggcagccgtcccctggagcttttcctgagcctgctgcgaaaccacgtcatccggatcgggggcaggtcctacgtccagtgtcaggggatcccacagggctccattctgtccacgctgctctgcagcctgtgctacggggacatggaaaacagactgtccccggggatccagcgtgacggggtgctcctgcgcttggtggacgacttcctgctggtgacccctcacctgacacgagccaaagcctttctcaggaccctggtccgcggcgtgcccgagtacggctgcctggccaacttgcggaagacggccgtgaacttccctgtggaggacggcgcccggggcggcccggccccactgcagctgccggcacactgcctgttcccctggtgcgggctgctgctggacacccgcacgctggaggtgcactgcgactatgccagttacgcccggacctcgatcagagcgagtctcaccttcaaccagggcttcaagcccgggaggaacatgcgccgcaagctcttggcggtcttgcggctaaagtgccacgggatccttctggacctgcaggtgaacagtcttccgacggtgctcgccaacgtttacaagatcttcctgctgcaggcctacaggttccacgcgtgtgtgctgcagctgcccttccgtcagccgcttgcgaggaacccctcatttttcctccggcttgtctccgacaccgcgtcctgctgctactcgctcctgaaagccagaaacgcagggatgtccctgggagccaggggcgcctccggcccgtttccctctgaagccgcagagtggctctgcctccacgccttcctgctcaagctggttcgtcaccgcgttacctacagctgtcttctggggccgctccgggcagccagagagcgattgtgccagcggctccctggggccacactggccgccctcgaggccgccgccgacccagccctgactacagacttccggaccatcctggactga

SEQ ID NO: 9 - DNA, 981 bp, Homo sapiens
  gene (1)..(981): hbmi1
atgcatcgaacaacgagaatcaagatcactgagctaaatccccacctgatgtgtgtgctttgtggagggtacttcattgatgccacaaccataatagaatgtctacattccttctgtaaaacgtgtattgttcgttacctggagaccagcaagtattgtcctatttgtgatgtccaagttcacaagaccagaccactactgaatataaggtcagataaaactctccaagatattgtatacaaattagttccagggcttttcaaaaatgaaatgaagagaagaagggatttttatgcagctcatccttctgctgatgctgccaatggctctaatgaagatagaggagaggttgcagatgaagataagagaattataactgatgatgagataataagcttatccattgaattctttgaccagaacagattggatcggaaagtaaacaaagacaaagagaaatctaaggaggaggtgaatgataaaagatacttacgatgcccagcagcaatgactgtgatgcacttaagaaagtttctcagaagtaaaatggacatacctaatactttccagattgatgtcatgtatgaggaggaacctttaaaggattattatacactaatggatattgcctacatttatacctggagaaggaatggtccacttccattgaaatacagagttcgacctacttgtaaaagaatgaagatcagtcaccagagagatggactgacaaatgctggagaactggaaagtgactctgggagtgacaaggccaacagcccagcaggaggtattccctccacctcttcttgtttgcctagccccagtactccagtgcagtctcctcatccacagtttcctcacatttccagtactatgaatggaaccagcaacagccccagcggtaaccaccaatcttcttttgccaatagacctcgaaaatcatcagtaaatgggtcatcagcaacttcttctggttga

SEQ ID NO: 10 - DNA, 20 bp, Artificial Sequence
  a primer for real-time PCR
ggcactgccctcagacttca

SEQ ID NO: 11 - DNA, 20 bp, Artificial Sequence
  a primer for real-time PCR
ctgctaaagcgcatgctcca

SEQ ID NO: 12 - DNA, 19 bp, Artificial Sequence
  a primer for real-time PCR
ctgcggcatccacgaacta

SEQ ID NO: 13 - DNA, 19 bp, Artificial Sequence
  a primer for real-time PCR
acagcaccgtgttggcgta

SEQ ID NO: 14 - DNA, 24 bp, Artificial Sequence
  a primer for real-time PCR
ttggtcaagcagcataatccaaag

SEQ ID NO: 15 - DNA, 23 bp, Artificial Sequence
  a primer for real-time PCR
gtcaagggcatagcctaccacaa

SEQ ID NO: 16 - DNA, 22 bp, Artificial Sequence
  a primer for real-time PCR
gcactgccctcagacttcaaga

SEQ ID NO: 17 - DNA, 20 bp, Artificial Sequence
  a primer for real-time PCR
gcgggactatggttgctgac

SEQ ID NO: 18 - DNA, 19 bp, Artificial Sequence
  a primer for real-time PCR
tggcacccagcacaatgaa

SEQ ID NO: 19 - DNA, 26 bp, Artificial Sequence
  a primer for real-time PCR
ctaagtcatagtccgcctagaagcca